European Patent Application EP 4 357 451 A1, published April 24, 2024. Title: Enzyme agent containing transglutaminase and its use. Applicant: AMANO ENZYME INC. The sequence listing filed with the application follows.

SEQUENCE LISTING (4 sequences)

SEQ ID NO: 1 - protein, 229 aa, Longimycelium tulufanense
ATSLPPIAPPLPRGVQSKSWSVPDYIAAWEKQHGRPMTAEERYHLARGCIGVTVVNLDREDAPNPPLNLSFGTYQRAMEVQAALNEIVATRPSPREYAEQVRKHPALQGVQNLVRAFPTFIDPANLHAAIFSKRFYSKQDPNWTDEQAAEMYRPNPRTGQVDMSTYRYRARPGYVNFDYGWYDEQTNNWWHANHAEPGMKVYQSTLRYYSRPLLDFDEQVFTVAFARVA

SEQ ID NO: 2 - protein, 265 aa, Longimycelium tulufanense
MKKWLPRALVALFVLLGLPAGLAGTAHAAVVAHAAVATSLPPIAPPLPRGVQSKSWSVPDYIAAWEKQHGRPMTAEERYHLARGCIGVTVVNLDREDAPNPPLNLSFGTYQRAMEVQAALNEIVATRPSPREYAEQVRKHPALQGVQNLVRAFPTFIDPANLHAAIFSKRFYSKQDPNWTDEQAAEMYRPNPRTGQVDMSTYRYRARPGYVNFDYGWYDEQTNNWWHANHAEPGMKVYQSTLRYYSRPLLDFDEQVFTVAFARVA

SEQ ID NO: 3 - DNA, 690 bp, Longimycelium tulufanense
gccacgtcgctgccaccgatcgcaccgccgcttccccggggcgtgcagagcaagagctggtcggtgccggactacattgccgcctgggagaagcaacacggtaggccgatgacggccgaggagcggtaccacctcgcccggggctgcatcggcgtcaccgtggtcaacctcgaccgggaggacgcgccgaacccgccgctcaacctgtcgttcggcacttaccagcgggccatggaagtgcaggccgcgctgaacgagatcgtcgcgacccggccgtcgccgcgggagtacgccgagcaggtgcgcaagcacccggcgctgcagggcgtgcagaacctggtgcgggcgttccccacgttcatcgacccggcgaacctgcacgccgccatcttctccaagcggttctactcgaagcaggacccgaactggaccgacgagcaggcggccgagatgtaccggccgaatccgcggaccggccaggtcgacatgagcacctaccgctaccgggcgcggccgggttacgtgaacttcgactacggttggtacgacgagcagacgaacaactggtggcacgccaaccacgcggagccgggcatgaaggtctaccagagcacgttgcggtactactcccggccgctgctggatttcgacgagcaggttttcaccgtggcgttcgcgcgggtcgcctga

SEQ ID NO: 4 - DNA, 798 bp, Longimycelium tulufanense
gtgaagaagtggttgccgcgcgccctggtcgcgctgttcgtgctcctggggttacccgccggcctggccggaacggcacatgccgcggtcgtcgcgcacgccgccgtcgccacgtcgctgccaccgatcgcaccgccgcttccccggggcgtgcagagcaagagctggtcggtgccggactacattgccgcctgggagaagcaacacggtaggccgatgacggccgaggagcggtaccacctcgcccggggctgcatcggcgtcaccgtggtcaacctcgaccgggaggacgcgccgaacccgccgctcaacctgtcgttcggcacttaccagcgggccatggaagtgcaggccgcgctgaacgagatcgtcgcgacccggccgtcgccgcgggagtacgccgagcaggtgcgcaagcacccggcgctgcagggcgtgcagaacctggtgcgggcgttccccacgttcatcgacccggcgaacctgcacgccgccatcttctccaagcggttctactcgaagcaggacccgaactggaccgacgagcaggcggccgagatgtaccggccgaatccgcggaccggccaggtcgacatgagcacctaccgctaccgggcgcggccgggttacgtgaacttcgactacggttggtacgacgagcagacgaacaactggtggcacgccaaccacgcggagccgggcatgaaggtctaccagagcacgttgcggtactactcccggccgctgctggatttcgacgagcaggttttcaccgtggcgttcgcgcgggtcgcctga